European Patent Application EP 4 477 231 A2, published December 18, 2024. Title: Combination vaccine. Applicant: CureVac SE. Application EP. The sequence listing filed with the application follows.

SEQUENCE LISTING (26 sequences)

SEQ ID NO: 1 - protein, 574 aa, Human respiratory syncytial virus
MELPILKANAITTILAAVTFCFASSQNITEEFYQSTCSAVSKGYLSALRTGWYTSVITIELSNIKENKCNGTDAKVKLINQELDKYKNAVTELQLLMQSTTAANNRARRELPRFMNYTLNNTKKTNVTLSKKRKRRFLGFLLGVGSAIASGIAVSKVLHLEGEVNKIKSALLSTNKAVVSLSNGVSVLTSKVLDLKNYIDKQLLPIVNKQSCRISNIETVIEFQQKNNRLLEITREFSVNAGVTTPVSTYMLTNSELLSLINDMPITNDQKKLMSNNVQIVRQQSYSIMSIIKEEVLAYVVQLPLYGVIDTPCWKLHTSPLCTTNTKEGSNICLTRTDRGWYCDNAGSVSFFPQAETCKVQSNRVFCDTMNSLTLPSEVNLCNVDIFNPKYDCKIMTSKTDVSSSVITSLGAIVSCYGKTKCTASNKNRGIIKTFSNGCDYVSNKGVDTVSVGNTLYYVNKQEGKSLYVKGEPIINFYDPLVFPSDEFDASISQVNEKINQSLAFIRKSDELLHHVNAGKSTTNIMITTIIIVIIVILLSLIAVGLLLYCKARSTPVTLSKDQLSGINNIAFSN

SEQ ID NO: 2 - protein, 574 aa, Human respiratory syncytial virus
MELLILKANAITTILTAVTFCFASGQNITEEFYQSTCSAVSKGYLSALRTGWYTSVITIELSNIKENKCNGTDAKVKLIKQELDKYKNAVTELQLLMQSTPPTNNRARRELPRFMNYTLNNAKKTNVTLSKKRKRRFLGFLLGVGSAIASGVAVSKVLHLEGEVNKIKSALLSTNKAVVSLSNGVSVLTSKVLDLKNYIDKQLLPIVNKQSCSISNIETVIEFQQKNNRLLEITREFSVNAGVTTPVSTYMLTNSELLSLINDMPITNDQKKLMSNNVQIVRQQSYSIMSIIKEEVLAYVVQLPLYGVIDTPCWKLHTSPLCTTNTKEGSNICLTRTDRGWYCDNAGSVSFFPQAETCKVQSNRVFCDTMNSLTLPSEINLCNVDIFNPKYDCKIMTSKTDVSSSVITSLGAIVSCYGKTKCTASNKNRGIIKTFSNGCDYVSNKGMDTVSVGNTLYYVNKQEGKSLYVKGEPIINFYDPLVFPSDEFDASISQVNEKINQSLAFIRKSDELLHNVNAGKSTTNIMITTIIIVIIVILLSLIAVGLLLYCKARSTPVTLSKDQLSGINNIAFSN

SEQ ID NO: 3 - protein, 565 aa, Influenza A virus
MKANLLVLLCALAAADADTICIGYHANNSTDTVDTVLEKNVTVTHSVNLLEDSHNGKLCRLKGIAPLQLGKCNIAGWLLGNPECDPLLPVRSWSYIVETPNSENGICYPGDFIDYEELREQLSSVSSFERFEIFPKESSWPNHNTNGVTAACSHEGKSSFYRNLLWLTEKEGSYPKLKNSYVNKKGKEVLVLWGIHHPPNSKEQQNLYQNENAYVSVVTSNYNRRFTPEIAERPKVRDQAGRMNYYWTLLKPGDTIIFEANGNLIAPMYAFALSRGFGSGIITSNASMHECNTKCQTPLGAINSSLPYQNIHPVTIGECPKYVRSAKLRMVTGLRNIPSIQSRGLFGAIAGFIEGGWTGMIDGWYGYHHQNEQGSGYAADQKSTQNAINGITNKVNTVIEKMNIQFTAVGKEFNKLEKRMENLNKKVDDGFLDIWTYNAELLVLLENERTLDFHDSNVKNLYEKVKSQLKNNAKEIGNGCFEFYHKCDNECMESVRNGTYDYPKYSEESKLNREKVDGVKLESMGIYQILAIYSTVASSLVLLVSLGAISFWMCSNGSLQCRICI

SEQ ID NO: 4 - DNA, 1725 bp, Human respiratory syncytial virus
  source 1..1725: mol_type = unassigned DNA
atggagttgccaatcctcaaagcaaatgcaattaccacaatcctcgctgcagtcacattttgctttgcttctagtcaaaacatcactgaagaattttatcaatcaacatgcagtgcagttagcaaaggctatcttagtgctctaagaactggttggtatactagtgttataactatagaattaagtaatatcaaggaaaataagtgtaatggaacagatgctaaggtaaaattgataaaccaagaattagataaatataaaaatgctgtaacagaattgcagttgctcatgcaaagcacaacagcagcaaacaatcgagccagaagagaactaccaaggtttatgaattatacactcaacaataccaaaaaaaccaatgtaacattaagcaagaaaaggaaaagaagatttcttggttttttgttaggtgttggatctgcaatcgccagtggcattgctgtatctaaggtcctgcacttagaaggagaagtgaacaagatcaaaagtgctctactatccacaaacaaggccgtagtcagcttatcaaatggagttagtgtcttaaccagcaaagtgttagacctcaaaaactatatagataaacaattgttacctattgtgaataagcaaagctgcagaatatcaaatatagaaactgtgatagagttccaacaaaagaacaacagactactagagattaccagggaatttagtgttaatgcaggtgtaactacacctgtaagcacttacatgttaactaatagtgaattattgtcattaatcaatgatatgcctataacaaatgatcagaaaaagttaatgtccaacaatgttcaaatagttagacagcaaagttactctatcatgtccataataaaagaggaagtcttagcatatgtagtacaattaccactatatggtgtgatagatacaccttgttggaaattacacacatcccctctatgtacaaccaacacaaaagaagggtcaaacatctgtttaacaagaactgacagaggatggtactgtgacaatgcaggatcagtatctttcttcccacaagctgaaacatgtaaagttcaatcgaatcgagtattttgtgacacaatgaacagtttaacattaccaagtgaagtaaatctctgcaatgttgacatattcaatcccaaatatgattgtaaaattatgacttcaaaaacagatgtaagcagctccgttatcacatctctaggagccattgtgtcatgctatggcaaaactaaatgtacagcatccaataaaaatcgtggaatcataaagacattttctaacgggtgtgattatgtatcaaataaaggggtggacactgtgtctgtaggtaacacattatattatgtaaataagcaagaaggcaaaagtctctatgtaaaaggtgaaccaataataaatttctatgacccattagtattcccctctgatgaatttgatgcatcaatatctcaagtcaatgagaagattaaccagagtttagcatttattcgtaaatccgatgaattattacatcatgtaaatgctggtaaatcaaccacaaatatcatgataactactataattatagtgattatagtaatattgttatcattaattgctgttggactgctcctatactgtaaggccagaagcacaccagtcacactaagcaaggatcaactgagtggtataaataatattgcatttagtaactga

SEQ ID NO: 5 - DNA, 1725 bp, Human respiratory syncytial virus
  source 1..1725: mol_type = unassigned DNA
atggagttgctaatcctcaaagcaaatgcaattaccacaatcctcactgcagtcacattttgttttgcttctggtcaaaacatcactgaagaattttatcaatcaacatgcagtgcagttagcaaaggctatcttagtgctctgagaactggttggtataccagtgttataactatagaattaagtaatatcaaggaaaataagtgtaatggaacagatgctaaggtaaaattgataaaacaagaattagataaatataaaaatgctgtaacagaattgcagttgctcatgcaaagcacaccaccaacaaacaatcgagccagaagagaactaccaaggtttatgaattatacactcaacaatgccaaaaaaaccaatgtaacattaagcaagaaaaggaaaagaagatttcttggttttttgttaggtgttggatctgcaatcgccagtggcgttgctgtatctaaggtcctgcacctagaaggggaagtgaacaagatcaaaagtgctctactatccacaaacaaggctgtagtcagcttatcaaatggagttagtgtcttaaccagcaaagtgttagacctcaaaaactatatagataaacaattgttacctattgtgaacaagcaaagctgcagcatatcaaatatagaaactgtgatagagttccaacaaaagaacaacagactactagagattaccagggaatttagtgttaatgcaggtgtaactacacctgtaagcacttacatgttaactaatagtgaattattgtcattaatcaatgatatgcctataacaaatgatcagaaaaagttaatgtccaacaatgttcaaatagttagacagcaaagttactctatcatgtccataataaaagaggaagtcttagcatatgtagtacaattaccactatatggtgttatagatacaccctgttggaaactacacacatcccctctatgtacaaccaacacaaaagaagggtccaacatctgtttaacaagaactgacagaggatggtactgtgacaatgcaggatcagtatctttcttcccacaagctgaaacatgtaaagttcaatcaaatcgagtattttgtgacacaatgaacagtttaacattaccaagtgaaataaatctctgcaatgttgacatattcaaccccaaatatgattgtaaaattatgacttcaaaaacagatgtaagcagctccgttatcacatctctaggagccattgtgtcatgctatggcaaaactaaatgtacagcatccaataaaaatcgtggaatcataaagacattttctaacgggtgcgattatgtatcaaataaagggatggacactgtgtctgtaggtaacacattatattatgtaaataagcaagaaggtaaaagtctctatgtaaaaggtgaaccaataataaatttctatgacccattagtattcccctctgatgaatttgatgcatcaatatctcaagtcaacgagaagattaaccagagcctagcatttattcgtaaatccgatgaattattacataatgtaaatgctggtaaatccaccacaaatatcatgataactactataattatagtgattatagtaatattgttatcattaattgctgttggactgctcttatactgtaaggccagaagcacaccagtcacactaagcaaagatcaactgagtggtataaataatattgcatttagtaactaa

SEQ ID NO: 6 - DNA, 1698 bp, Influenza A virus
  source 1..1698: mol_type = unassigned DNA
atgaaggcaaacctactggtcctgttatgtgcacttgcagctgcagatgcagacacaatatgtataggctaccatgcgaacaattcaaccgacactgttgacacagtactcgagaagaatgtgacagtgacacactctgttaacctgctcgaagacagccacaacggaaaactatgtagattaaaaggaatagccccactacaattggggaaatgtaacatcgccggatggctcttgggaaacccagaatgcgacccactgcttccagtgagatcatggtcctacattgtagaaacaccaaactctgagaatggaatatgttatccaggagatttcatcgactatgaggagctgagggagcaattgagctcagtgtcatcattcgaaagattcgaaatatttcccaaagaaagctcatggcccaaccacaacacaaacggagtaacggcagcatgctcccatgaggggaaaagcagtttttacagaaatttgctatggctgacggagaaggagggctcatacccaaagctgaaaaattcttatgtgaacaaaaaagggaaagaagtccttgtactgtggggtattcatcacccgcctaacagtaaggaacaacagaatctctatcagaatgaaaatgcttatgtctctgtagtgacttcaaattataacaggagatttaccccggaaatagcagaaagacccaaagtaagagatcaagctgggaggatgaactattactggaccttgctaaaacccggagacacaataatatttgaggcaaatggaaatctaatagcaccaatgtatgctttcgcactgagtagaggctttgggtccggcatcatcacctcaaacgcatcaatgcatgagtgtaacacgaagtgtcaaacacccctgggagctataaacagcagtctcccttaccagaatatacacccagtcacaataggagagtgcccaaaatacgtcaggagtgccaaattgaggatggttacaggactaaggaacaatccgtccattcaatccagaggtctatttggagccattgccggttttattgaagggggatggactggaatgatagatggatggtatggttatcatcatcagaatgaacagggatcaggctatgcagcggatcaaaaaagcacacaaaatgccattaacgggattacaaacaaggtgaacactgttatcgagaaaatgaacattcaattcacagctgtgggtaaagaattcaacaaattagaaaaaaggatggaaaatttaaataaaaaagttgatgatggatttctggacatttggacatataatgcagaattgttagttctactggaaaatgaaaggactctggatttccatgactcaaatgtgaagaatctgtatgagaaagtaaaaagccaattaaagaataatgccaaagaaatcggaaatggatgttttgagttctaccacaagtgtgacaatgaatgcatggaaagtgtaagaaatgggacttatgattatcccaaatattcagaagagtcaaagttgaacagggaaaaggtagatggagtgaaattggaatcaatggggatctatcagattctggcgatctactcaactgtcgccagttcactggtgcttttggtctccctgggggcaatcagtttctggatgtgttctaatggatctttgcagtgcagaatatgcatctga

SEQ ID NO: 7 - DNA, 1725 bp, synthetic construct
  misc_feature 1..1725: note = GC-enriched DNA coding sequence coding for the Fusion (F) protein of RSV Long
  source 1..1725: mol_type = other DNA
atggagctgcccatcctcaaggccaacgccatcaccaccatcctggcggccgtgacgttctgcttcgccagctcccagaacatcaccgaggagttctaccagagcacctgctccgccgtcagcaagggctacctgtccgccctccggaccgggtggtacacgagcgtgatcaccatcgagctgtccaacatcaaggagaacaagtgcaacggcaccgacgcgaaggtgaagctgatcaaccaggagctcgacaagtacaagaacgccgtcaccgagctgcagctgctcatgcagagcacgaccgccgccaacaaccgcgcgcggcgcgagctgccgcggttcatgaactacaccctgaacaacaccaagaagacgaacgtgaccctctccaagaagcgcaagcggcgcttcctggggttcctgctcggcgtggggagcgccatcgcctccggcatcgccgtcagcaaggtgctgcacctggagggcgaggtgaacaagatcaagtccgccctcctgagcaccaacaaggcggtcgtgtccctgagcaacggggtgtccgtcctcaccagcaaggtgctggacctgaagaactacatcgacaagcagctcctgcccatcgtgaacaagcagtcctgccggatcagcaacatcgagacggtcatcgagttccagcagaagaacaaccgcctgctcgagatcacccgggagttcagcgtgaacgccggcgtgaccacccccgtctccacgtacatgctgaccaacagcgagctgctctccctgatcaacgacatgcccatcaccaacgaccagaagaagctgatgagcaacaacgtgcagatcgtgcgccagcagtcctacagcatcatgtccatcatcaaggaggaggtcctcgcctacgtggtgcagctgccgctgtacggggtcatcgacaccccctgctggaagctccacacgagccccctgtgcaccaccaacaccaaggagggctccaacatctgcctgacgcggaccgaccgcgggtggtactgcgacaacgccggcagcgtgtccttcttcccccaggccgagacctgcaaggtccagagcaaccgggtgttctgcgacaccatgaactccctcacgctgccgagcgaggtgaacctgtgcaacgtcgacatcttcaaccccaagtacgactgcaagatcatgacctccaagaccgacgtgagctccagcgtgatcacctccctcggcgcgatcgtcagctgctacgggaagacgaagtgcaccgccagcaacaagaaccgcggcatcatcaagaccttctccaacgggtgcgactacgtgagcaacaagggcgtggacaccgtctccgtgggcaacaccctgtactacgtgaacaagcaggaggggaagagcctgtacgtcaagggcgagcccatcatcaacttctacgaccccctcgtgttcccgtccgacgagttcgacgccagcatctcccaggtgaacgagaagatcaaccagagcctggccttcatccggaagtccgacgagctgctgcaccacgtcaacgccgggaagagcacgaccaacatcatgatcaccaccatcatcatcgtgatcatcgtgatcctcctgtccctgatcgcggtcggcctcctgctgtactgcaaggcccgcagcacgcccgtgaccctctccaaggaccagctgagcgggatcaacaacatcgccttctccaactga

SEQ ID NO: 8 - DNA, 1725 bp, synthetic construct
  misc_feature 1..1725: note = GC-enriched DNA coding sequence coding for the Fusion (F) protein of RSV A2
  source 1..1725: mol_type = other DNA
atggagctgctcatcctgaaggccaacgccatcaccaccatcctgacggcggtgaccttctgcttcgccagcggccagaacatcaccgaggagttctaccagtccacctgcagcgccgtctccaaggggtacctcagcgccctgcggacgggctggtacacctccgtgatcaccatcgagctgagcaacatcaaggagaacaagtgcaacgggaccgacgccaaggtgaagctcatcaagcaggagctggacaagtacaagaacgcggtcacggagctgcagctcctgatgcagtccaccccgccgaccaacaaccgcgcccggcgcgagctgccccggttcatgaactacaccctcaacaacgccaagaagacgaacgtgaccctgagcaagaagcgcaagcggcgcttcctgggcttcctcctgggggtgggctccgccatcgcgagcggcgtcgccgtgtccaaggtgctgcacctcgagggggaggtcaacaagatcaagagcgccctgctgtccaccaacaaggccgtggtgagcctctccaacggcgtcagcgtgctgacctccaaggtgctggacctcaagaactacatcgacaagcagctgctgcccatcgtcaacaagcagagctgctccatcagcaacatcgagacggtgatcgagttccagcagaagaacaaccggctcctggagatcacccgcgagttcagcgtgaacgccggggtcaccacccccgtgtccacgtacatgctgaccaacagcgagctcctgtccctgatcaacgacatgccgatcaccaacgaccagaagaagctcatgagcaacaacgtgcagatcgtccggcagcagtcctacagcatcatgtccatcatcaaggaggaggtgctggcgtacgtggtccagctgcccctctacggcgtgatcgacaccccctgctggaagctgcacacgagccccctgtgcaccaccaacaccaaggaggggtccaacatctgcctcacgcgcaccgaccggggctggtactgcgacaacgccggcagcgtctccttcttcccgcaggccgagacctgcaaggtgcagagcaaccgcgtgttctgcgacaccatgaactccctgacgctgcccagcgagatcaacctctgcaacgtcgacatcttcaaccccaagtacgactgcaagatcatgacctccaagaccgacgtgagctccagcgtgatcacctccctgggggccatcgtcagctgctacggcaagacgaagtgcaccgccagcaacaagaaccgggggatcatcaagaccttctccaacggctgcgactacgtgagcaacaagggcatggacaccgtgtccgtcgggaacaccctgtactacgtgaacaagcaggagggcaagagcctctacgtgaagggggagcccatcatcaacttctacgacccgctggtcttcccctccgacgagttcgacgcgagcatctcccaggtgaacgagaagatcaaccagagcctggccttcatccgcaagtccgacgagctgctccacaacgtgaacgccggcaagagcacgaccaacatcatgatcaccaccatcatcatcgtcatcatcgtgatcctgctgtccctcatcgccgtggggctgctgctctactgcaaggcccggagcacgcccgtcaccctgtccaaggaccagctgagcggcatcaacaacatcgcgttctccaactga

SEQ ID NO: 9 - DNA, 1725 bp, synthetic construct
  misc_feature 1..1725: note = GC-enriched DNA coding sequence coding for the Fusion (F) protein of RSV A2 (P102A)
  source 1..1725: mol_type = other DNA
atggagctgctcatcctgaaggccaacgccatcaccaccatcctgacggcggtgaccttctgcttcgccagcggccagaacatcaccgaggagttctaccagtccacctgcagcgccgtctccaaggggtacctcagcgccctgcggacgggctggtacacctccgtgatcaccatcgagctgagcaacatcaaggagaacaagtgcaacgggaccgacgccaaggtgaagctcatcaagcaggagctggacaagtacaagaacgcggtcacggagctgcagctcctgatgcagtccaccccggcgaccaacaaccgcgcccggcgcgagctgccccggttcatgaactacaccctcaacaacgccaagaagacgaacgtgaccctgagcaagaagcgcaagcggcgcttcctgggcttcctcctgggggtgggctccgccatcgcgagcggcgtcgccgtgtccaaggtgctgcacctcgagggggaggtcaacaagatcaagagcgccctgctgtccaccaacaaggccgtggtgagcctctccaacggcgtcagcgtgctgacctccaaggtgctggacctcaagaactacatcgacaagcagctgctgcccatcgtcaacaagcagagctgctccatcagcaacatcgagacggtgatcgagttccagcagaagaacaaccggctcctggagatcacccgcgagttcagcgtgaacgccggggtcaccacccccgtgtccacgtacatgctgaccaacagcgagctcctgtccctgatcaacgacatgccgatcaccaacgaccagaagaagctcatgagcaacaacgtgcagatcgtccggcagcagtcctacagcatcatgtccatcatcaaggaggaggtgctggcgtacgtggtccagctgcccctctacggcgtgatcgacaccccctgctggaagctgcacacgagccccctgtgcaccaccaacaccaaggaggggtccaacatctgcctcacgcgcaccgaccggggctggtactgcgacaacgccggcagcgtctccttcttcccgcaggccgagacctgcaaggtgcagagcaaccgcgtgttctgcgacaccatgaactccctgacgctgcccagcgagatcaacctctgcaacgtcgacatcttcaaccccaagtacgactgcaagatcatgacctccaagaccgacgtgagctccagcgtgatcacctccctgggggccatcgtcagctgctacggcaagacgaagtgcaccgccagcaacaagaaccgggggatcatcaagaccttctccaacggctgcgactacgtgagcaacaagggcatggacaccgtgtccgtcgggaacaccctgtactacgtgaacaagcaggagggcaagagcctctacgtgaagggggagcccatcatcaacttctacgacccgctggtcttcccctccgacgagttcgacgcgagcatctcccaggtgaacgagaagatcaaccagagcctggccttcatccgcaagtccgacgagctgctccacaacgtgaacgccggcaagagcacgaccaacatcatgatcaccaccatcatcatcgtcatcatcgtgatcctgctgtccctcatcgccgtggggctgctgctctactgcaaggcccggagcacgcccgtcaccctgtccaaggaccagctgagcggcatcaacaacatcgcgttctccaactga

SEQ ID NO: 10 - DNA, 1725 bp, synthetic construct
  misc_feature 1..1725: note = GC-enriched DNA coding sequence coding for the Fusion (F) protein of RSV A2 (I379V)
  source 1..1725: mol_type = other DNA
atggagctgctcatcctgaaggccaacgccatcaccaccatcctgacggcggtgaccttctgcttcgccagcggccagaacatcaccgaggagttctaccagtccacctgcagcgccgtctccaaggggtacctcagcgccctgcggacgggctggtacacctccgtgatcaccatcgagctgagcaacatcaaggagaacaagtgcaacgggaccgacgccaaggtgaagctcatcaagcaggagctggacaagtacaagaacgcggtcacggagctgcagctcctgatgcagtccaccccgccgaccaacaaccgcgcccggcgcgagctgccccggttcatgaactacaccctcaacaacgccaagaagacgaacgtgaccctgagcaagaagcgcaagcggcgcttcctgggcttcctcctgggggtgggctccgccatcgcgagcggcgtcgccgtgtccaaggtgctgcacctcgagggggaggtcaacaagatcaagagcgccctgctgtccaccaacaaggccgtggtgagcctctccaacggcgtcagcgtgctgacctccaaggtgctggacctcaagaactacatcgacaagcagctgctgcccatcgtcaacaagcagagctgctccatcagcaacatcgagacggtgatcgagttccagcagaagaacaaccggctcctggagatcacccgcgagttcagcgtgaacgccggggtcaccacccccgtgtccacgtacatgctgaccaacagcgagctcctgtccctgatcaacgacatgccgatcaccaacgaccagaagaagctcatgagcaacaacgtgcagatcgtccggcagcagtcctacagcatcatgtccatcatcaaggaggaggtgctggcgtacgtggtccagctgcccctctacggcgtgatcgacaccccctgctggaagctgcacacgagccccctgtgcaccaccaacaccaaggaggggtccaacatctgcctcacgcgcaccgaccggggctggtactgcgacaacgccggcagcgtctccttcttcccgcaggccgagacctgcaaggtgcagagcaaccgcgtgttctgcgacaccatgaactccctgacgctgcccagcgaggtcaacctctgcaacgtcgacatcttcaaccccaagtacgactgcaagatcatgacctccaagaccgacgtgagctccagcgtgatcacctccctgggggccatcgtcagctgctacggcaagacgaagtgcaccgccagcaacaagaaccgggggatcatcaagaccttctccaacggctgcgactacgtgagcaacaagggcatggacaccgtgtccgtcgggaacaccctgtactacgtgaacaagcaggagggcaagagcctctacgtgaagggggagcccatcatcaacttctacgacccgctggtcttcccctccgacgagttcgacgcgagcatctcccaggtgaacgagaagatcaaccagagcctggccttcatccgcaagtccgacgagctgctccacaacgtgaacgccggcaagagcacgaccaacatcatgatcaccaccatcatcatcgtcatcatcgtgatcctgctgtccctcatcgccgtggggctgctgctctactgcaaggcccggagcacgcccgtcaccctgtccaaggaccagctgagcggcatcaacaacatcgcgttctccaactga

SEQ ID NO: 11 - DNA, 1725 bp, synthetic construct
  misc_feature 1..1725: note = GC-enriched DNA coding sequence coding for the Fusion (F) protein of RSV A2 (M447V)
  source 1..1725: mol_type = other DNA
atggagctgctcatcctgaaggccaacgccatcaccaccatcctgacggcggtgaccttctgcttcgccagcggccagaacatcaccgaggagttctaccagtccacctgcagcgccgtctccaaggggtacctcagcgccctgcggacgggctggtacacctccgtgatcaccatcgagctgagcaacatcaaggagaacaagtgcaacgggaccgacgccaaggtgaagctcatcaagcaggagctggacaagtacaagaacgcggtcacggagctgcagctcctgatgcagtccaccccgccgaccaacaaccgcgcccggcgcgagctgccccggttcatgaactacaccctcaacaacgccaagaagacgaacgtgaccctgagcaagaagcgcaagcggcgcttcctgggcttcctcctgggggtgggctccgccatcgcgagcggcgtcgccgtgtccaaggtgctgcacctcgagggggaggtcaacaagatcaagagcgccctgctgtccaccaacaaggccgtggtgagcctctccaacggcgtcagcgtgctgacctccaaggtgctggacctcaagaactacatcgacaagcagctgctgcccatcgtcaacaagcagagctgctccatcagcaacatcgagacggtgatcgagttccagcagaagaacaaccggctcctggagatcacccgcgagttcagcgtgaacgccggggtcaccacccccgtgtccacgtacatgctgaccaacagcgagctcctgtccctgatcaacgacatgccgatcaccaacgaccagaagaagctcatgagcaacaacgtgcagatcgtccggcagcagtcctacagcatcatgtccatcatcaaggaggaggtgctggcgtacgtggtccagctgcccctctacggcgtgatcgacaccccctgctggaagctgcacacgagccccctgtgcaccaccaacaccaaggaggggtccaacatctgcctcacgcgcaccgaccggggctggtactgcgacaacgccggcagcgtctccttcttcccgcaggccgagacctgcaaggtgcagagcaaccgcgtgttctgcgacaccatgaactccctgacgctgcccagcgagatcaacctctgcaacgtcgacatcttcaaccccaagtacgactgcaagatcatgacctccaagaccgacgtgagctccagcgtgatcacctccctgggggccatcgtcagctgctacggcaagacgaagtgcaccgccagcaacaagaaccgggggatcatcaagaccttctccaacggctgcgactacgtgagcaacaagggcgtggacaccgtgtccgtcgggaacaccctgtactacgtgaacaagcaggagggcaagagcctctacgtgaagggggagcccatcatcaacttctacgacccgctggtcttcccctccgacgagttcgacgcgagcatctcccaggtgaacgagaagatcaaccagagcctggccttcatccgcaagtccgacgagctgctccacaacgtgaacgccggcaagagcacgaccaacatcatgatcaccaccatcatcatcgtcatcatcgtgatcctgctgtccctcatcgccgtggggctgctgctctactgcaaggcccggagcacgcccgtcaccctgtccaaggaccagctgagcggcatcaacaacatcgcgttctccaactga

SEQ ID NO: 12 - DNA, 1698 bp, synthetic construct
  misc_feature 1..1698: note = GC-enriched DNA coding sequence coding for the Hemagglutinin (HA) protein of Influenza A/Puerto Rico/8/1934
  source 1..1698: mol_type = other DNA
atgaaggccaacctgctcgtgctgctgtgcgccctcgcggccgccgacgccgacaccatctgcatcggctaccacgccaacaacagcaccgacacggtcgacaccgtgctggagaagaacgtgaccgtcacccactccgtgaacctgctcgaggacagccacaacgggaagctgtgccggctgaagggcatcgcgcccctccagctggggaagtgcaacatcgccggctggctgctcgggaacccggagtgcgaccccctgctgcccgtgcgctcctggagctacatcgtcgagacgcccaactccgagaacggcatctgctacccgggcgacttcatcgactacgaggagctccgggagcagctgagctccgtgagctccttcgagcgcttcgagatcttccccaaggagagctcctggcccaaccacaacaccaacggggtgaccgccgcctgcagccacgagggcaagtccagcttctaccggaacctgctctggctgaccgagaaggaggggtcctaccccaagctgaagaacagctacgtcaacaagaagggcaaggaggtgctcgtgctgtgggggatccaccacccgcccaactccaaggagcagcagaacctgtaccagaacgagaacgcgtacgtcagcgtggtgacgtccaactacaaccgccggttcacccccgagatcgccgagcgccccaaggtccgggaccaggccggccgcatgaactactactggaccctcctgaagccgggcgacaccatcatcttcgaggccaacgggaacctgatcgccccgatgtacgcgttcgccctcagccggggcttcgggagcggcatcatcacgtccaacgccagcatgcacgagtgcaacaccaagtgccagacccccctgggcgccatcaactccagcctgccctaccagaacatccacccggtgaccatcggggagtgccccaagtacgtgcgctccgccaagctccggatggtcacgggcctgcgcaacaaccccagcatccagtcccgggggctgttcggcgcgatcgccgggttcatcgagggcggctggaccgggatgatcgacggctggtacgggtaccaccaccagaacgagcagggcagcgggtacgccgccgaccagaagtccacccagaacgccatcaacggcatcaccaacaaggtgaacacggtgatcgagaagatgaacatccagttcaccgcggtcggcaaggagttcaacaagctcgagaagcgcatggagaacctgaacaagaaggtggacgacgggttcctggacatctggacctacaacgccgagctcctggtgctgctcgagaacgagcggaccctggacttccacgacagcaacgtcaagaacctgtacgagaaggtgaagtcccagctcaagaacaacgccaaggagatcggcaacgggtgcttcgagttctaccacaagtgcgacaacgagtgcatggagagcgtccgcaacggcacgtacgactaccccaagtactccgaggagagcaagctgaaccgggagaaggtggacggggtgaagctggagtccatgggcatctaccagatcctcgccatctacagcaccgtcgcctccagcctggtgctgctggtgtccctcggcgcgatcagcttctggatgtgcagcaacgggtccctgcagtgccgcatctgcatctga

SEQ ID NO: 13 - RNA, 1725 nt, synthetic construct
  misc_feature 1..1725: note = GC-enriched RNA sequence without UTRs coding for the Fusion (F) protein of RSV Long
  source 1..1725: mol_type = other RNA
atggagctgcccatcctcaaggccaacgccatcaccaccatcctggcggccgtgacgttctgcttcgccagctcccagaacatcaccgaggagttctaccagagcacctgctccgccgtcagcaagggctacctgtccgccctccggaccgggtggtacacgagcgtgatcaccatcgagctgtccaacatcaaggagaacaagtgcaacggcaccgacgcgaaggtgaagctgatcaaccaggagctcgacaagtacaagaacgccgtcaccgagctgcagctgctcatgcagagcacgaccgccgccaacaaccgcgcgcggcgcgagctgccgcggttcatgaactacaccctgaacaacaccaagaagacgaacgtgaccctctccaagaagcgcaagcggcgcttcctggggttcctgctcggcgtggggagcgccatcgcctccggcatcgccgtcagcaaggtgctgcacctggagggcgaggtgaacaagatcaagtccgccctcctgagcaccaacaaggcggtcgtgtccctgagcaacggggtgtccgtcctcaccagcaaggtgctggacctgaagaactacatcgacaagcagctcctgcccatcgtgaacaagcagtcctgccggatcagcaacatcgagacggtcatcgagttccagcagaagaacaaccgcctgctcgagatcacccgggagttcagcgtgaacgccggcgtgaccacccccgtctccacgtacatgctgaccaacagcgagctgctctccctgatcaacgacatgcccatcaccaacgaccagaagaagctgatgagcaacaacgtgcagatcgtgcgccagcagtcctacagcatcatgtccatcatcaaggaggaggtcctcgcctacgtggtgcagctgccgctgtacggggtcatcgacaccccctgctggaagctccacacgagccccctgtgcaccaccaacaccaaggagggctccaacatctgcctgacgcggaccgaccgcgggtggtactgcgacaacgccggcagcgtgtccttcttcccccaggccgagacctgcaaggtccagagcaaccgggtgttctgcgacaccatgaactccctcacgctgccgagcgaggtgaacctgtgcaacgtcgacatcttcaaccccaagtacgactgcaagatcatgacctccaagaccgacgtgagctccagcgtgatcacctccctcggcgcgatcgtcagctgctacgggaagacgaagtgcaccgccagcaacaagaaccgcggcatcatcaagaccttctccaacgggtgcgactacgtgagcaacaagggcgtggacaccgtctccgtgggcaacaccctgtactacgtgaacaagcaggaggggaagagcctgtacgtcaagggcgagcccatcatcaacttctacgaccccctcgtgttcccgtccgacgagttcgacgccagcatctcccaggtgaacgagaagatcaaccagagcctggccttcatccggaagtccgacgagctgctgcaccacgtcaacgccgggaagagcacgaccaacatcatgatcaccaccatcatcatcgtgatcatcgtgatcctcctgtccctgatcgcggtcggcctcctgctgtactgcaaggcccgcagcacgcccgtgaccctctccaaggaccagctgagcgggatcaacaacatcgccttctccaactga

SEQ ID NO: 14 - RNA, 1725 nt, synthetic construct
  misc_feature 1..1725: note = GC-enriched RNA sequence without UTRs coding for the Fusion (F) protein of RSV A2
  source 1..1725: mol_type = other RNA
atggagctgctcatcctgaaggccaacgccatcaccaccatcctgacggcggtgaccttctgcttcgccagcggccagaacatcaccgaggagttctaccagtccacctgcagcgccgtctccaaggggtacctcagcgccctgcggacgggctggtacacctccgtgatcaccatcgagctgagcaacatcaaggagaacaagtgcaacgggaccgacgccaaggtgaagctcatcaagcaggagctggacaagtacaagaacgcggtcacggagctgcagctcctgatgcagtccaccccgccgaccaacaaccgcgcccggcgcgagctgccccggttcatgaactacaccctcaacaacgccaagaagacgaacgtgaccctgagcaagaagcgcaagcggcgcttcctgggcttcctcctgggggtgggctccgccatcgcgagcggcgtcgccgtgtccaaggtgctgcacctcgagggggaggtcaacaagatcaagagcgccctgctgtccaccaacaaggccgtggtgagcctctccaacggcgtcagcgtgctgacctccaaggtgctggacctcaagaactacatcgacaagcagctgctgcccatcgtcaacaagcagagctgctccatcagcaacatcgagacggtgatcgagttccagcagaagaacaaccggctcctggagatcacccgcgagttcagcgtgaacgccggggtcaccacccccgtgtccacgtacatgctgaccaacagcgagctcctgtccctgatcaacgacatgccgatcaccaacgaccagaagaagctcatgagcaacaacgtgcagatcgtccggcagcagtcctacagcatcatgtccatcatcaaggaggaggtgctggcgtacgtggtccagctgcccctctacggcgtgatcgacaccccctgctggaagctgcacacgagccccctgtgcaccaccaacaccaaggaggggtccaacatctgcctcacgcgcaccgaccggggctggtactgcgacaacgccggcagcgtctccttcttcccgcaggccgagacctgcaaggtgcagagcaaccgcgtgttctgcgacaccatgaactccctgacgctgcccagcgagatcaacctctgcaacgtcgacatcttcaaccccaagtacgactgcaagatcatgacctccaagaccgacgtgagctccagcgtgatcacctccctgggggccatcgtcagctgctacggcaagacgaagtgcaccgccagcaacaagaaccgggggatcatcaagaccttctccaacggctgcgactacgtgagcaacaagggcatggacaccgtgtccgtcgggaacaccctgtactacgtgaacaagcaggagggcaagagcctctacgtgaagggggagcccatcatcaacttctacgacccgctggtcttcccctccgacgagttcgacgcgagcatctcccaggtgaacgagaagatcaaccagagcctggccttcatccgcaagtccgacgagctgctccacaacgtgaacgccggcaagagcacgaccaacatcatgatcaccaccatcatcatcgtcatcatcgtgatcctgctgtccctcatcgccgtggggctgctgctctactgcaaggcccggagcacgcccgtcaccctgtccaaggaccagctgagcggcatcaacaacatcgcgttctccaactga

SEQ ID NO: 15 - RNA, 1725 nt, synthetic construct
  misc_feature 1..1725: note = GC-enriched RNA sequence without UTRs coding for the Fusion (F) protein of RSV A2 (P102A)
  source 1..1725: mol_type = other RNA
atggagctgctcatcctgaaggccaacgccatcaccaccatcctgacggcggtgaccttctgcttcgccagcggccagaacatcaccgaggagttctaccagtccacctgcagcgccgtctccaaggggtacctcagcgccctgcggacgggctggtacacctccgtgatcaccatcgagctgagcaacatcaaggagaacaagtgcaacgggaccgacgccaaggtgaagctcatcaagcaggagctggacaagtacaagaacgcggtcacggagctgcagctcctgatgcagtccaccccggcgaccaacaaccgcgcccggcgcgagctgccccggttcatgaactacaccctcaacaacgccaagaagacgaacgtgaccctgagcaagaagcgcaagcggcgcttcctgggcttcctcctgggggtgggctccgccatcgcgagcggcgtcgccgtgtccaaggtgctgcacctcgagggggaggtcaacaagatcaagagcgccctgctgtccaccaacaaggccgtggtgagcctctccaacggcgtcagcgtgctgacctccaaggtgctggacctcaagaactacatcgacaagcagctgctgcccatcgtcaacaagcagagctgctccatcagcaacatcgagacggtgatcgagttccagcagaagaacaaccggctcctggagatcacccgcgagttcagcgtgaacgccggggtcaccacccccgtgtccacgtacatgctgaccaacagcgagctcctgtccctgatcaacgacatgccgatcaccaacgaccagaagaagctcatgagcaacaacgtgcagatcgtccggcagcagtcctacagcatcatgtccatcatcaaggaggaggtgctggcgtacgtggtccagctgcccctctacggcgtgatcgacaccccctgctggaagctgcacacgagccccctgtgcaccaccaacaccaaggaggggtccaacatctgcctcacgcgcaccgaccggggctggtactgcgacaacgccggcagcgtctccttcttcccgcaggccgagacctgcaaggtgcagagcaaccgcgtgttctgcgacaccatgaactccctgacgctgcccagcgagatcaacctctgcaacgtcgacatcttcaaccccaagtacgactgcaagatcatgacctccaagaccgacgtgagctccagcgtgatcacctccctgggggccatcgtcagctgctacggcaagacgaagtgcaccgccagcaacaagaaccgggggatcatcaagaccttctccaacggctgcgactacgtgagcaacaagggcatggacaccgtgtccgtcgggaacaccctgtactacgtgaacaagcaggagggcaagagcctctacgtgaagggggagcccatcatcaacttctacgacccgctggtcttcccctccgacgagttcgacgcgagcatctcccaggtgaacgagaagatcaaccagagcctggccttcatccgcaagtccgacgagctgctccacaacgtgaacgccggcaagagcacgaccaacatcatgatcaccaccatcatcatcgtcatcatcgtgatcctgctgtccctcatcgccgtggggctgctgctctactgcaaggcccggagcacgcccgtcaccctgtccaaggaccagctgagcggcatcaacaacatcgcgttctccaactga

SEQ ID NO: 16 - RNA, 1725 nt, synthetic construct
  misc_feature 1..1725: note = GC-enriched RNA sequence without UTRs coding for the Fusion (F) protein of RSV A2 (I379V)
  source 1..1725: mol_type = other RNA
atggagctgctcatcctgaaggccaacgccatcaccaccatcctgacggcggtgaccttctgcttcgccagcggccagaacatcaccgaggagttctaccagtccacctgcagcgccgtctccaaggggtacctcagcgccctgcggacgggctggtacacctccgtgatcaccatcgagctgagcaacatcaaggagaacaagtgcaacgggaccgacgccaaggtgaagctcatcaagcaggagctggacaagtacaagaacgcggtcacggagctgcagctcctgatgcagtccaccccgccgaccaacaaccgcgcccggcgcgagctgccccggttcatgaactacaccctcaacaacgccaagaagacgaacgtgaccctgagcaagaagcgcaagcggcgcttcctgggcttcctcctgggggtgggctccgccatcgcgagcggcgtcgccgtgtccaaggtgctgcacctcgagggggaggtcaacaagatcaagagcgccctgctgtccaccaacaaggccgtggtgagcctctccaacggcgtcagcgtgctgacctccaaggtgctggacctcaagaactacatcgacaagcagctgctgcccatcgtcaacaagcagagctgctccatcagcaacatcgagacggtgatcgagttccagcagaagaacaaccggctcctggagatcacccgcgagttcagcgtgaacgccggggtcaccacccccgtgtccacgtacatgctgaccaacagcgagctcctgtccctgatcaacgacatgccgatcaccaacgaccagaagaagctcatgagcaacaacgtgcagatcgtccggcagcagtcctacagcatcatgtccatcatcaaggaggaggtgctggcgtacgtggtccagctgcccctctacggcgtgatcgacaccccctgctggaagctgcacacgagccccctgtgcaccaccaacaccaaggaggggtccaacatctgcctcacgcgcaccgaccggggctggtactgcgacaacgccggcagcgtctccttcttcccgcaggccgagacctgcaaggtgcagagcaaccgcgtgttctgcgacaccatgaactccctgacgctgcccagcgaggtcaacctctgcaacgtcgacatcttcaaccccaagtacgactgcaagatcatgacctccaagaccgacgtgagctccagcgtgatcacctccctgggggccatcgtcagctgctacggcaagacgaagtgcaccgccagcaacaagaaccgggggatcatcaagaccttctccaacggctgcgactacgtgagcaacaagggcatggacaccgtgtccgtcgggaacaccctgtactacgtgaacaagcaggagggcaagagcctctacgtgaagggggagcccatcatcaacttctacgacccgctggtcttcccctccgacgagttcgacgcgagcatctcccaggtgaacgagaagatcaaccagagcctggccttcatccgcaagtccgacgagctgctccacaacgtgaacgccggcaagagcacgaccaacatcatgatcaccaccatcatcatcgtcatcatcgtgatcctgctgtccctcatcgccgtggggctgctgctctactgcaaggcccggagcacgcccgtcaccctgtccaaggaccagctgagcggcatcaacaacatcgcgttctccaactga

SEQ ID NO: 17 - RNA, 1725 nt, synthetic construct
  misc_feature 1..1725: note = GC-enriched RNA sequence without UTRs coding for the Fusion (F) protein of RSV A2 (M447V)
  source 1..1725: mol_type = other RNA
atggagctgctcatcctgaaggccaacgccatcaccaccatcctgacggcggtgaccttctgcttcgccagcggccagaacatcaccgaggagttctaccagtccacctgcagcgccgtctccaaggggtacctcagcgccctgcggacgggctggtacacctccgtgatcaccatcgagctgagcaacatcaaggagaacaagtgcaacgggaccgacgccaaggtgaagctcatcaagcaggagctggacaagtacaagaacgcggtcacggagctgcagctcctgatgcagtccaccccgccgaccaacaaccgcgcccggcgcgagctgccccggttcatgaactacaccctcaacaacgccaagaagacgaacgtgaccctgagcaagaagcgcaagcggcgcttcctgggcttcctcctgggggtgggctccgccatcgcgagcggcgtcgccgtgtccaaggtgctgcacctcgagggggaggtcaacaagatcaagagcgccctgctgtccaccaacaaggccgtggtgagcctctccaacggcgtcagcgtgctgacctccaaggtgctggacctcaagaactacatcgacaagcagctgctgcccatcgtcaacaagcagagctgctccatcagcaacatcgagacggtgatcgagttccagcagaagaacaaccggctcctggagatcacccgcgagttcagcgtgaacgccggggtcaccacccccgtgtccacgtacatgctgaccaacagcgagctcctgtccctgatcaacgacatgccgatcaccaacgaccagaagaagctcatgagcaacaacgtgcagatcgtccggcagcagtcctacagcatcatgtccatcatcaaggaggaggtgctggcgtacgtggtccagctgcccctctacggcgtgatcgacaccccctgctggaagctgcacacgagccccctgtgcaccaccaacaccaaggaggggtccaacatctgcctcacgcgcaccgaccggggctggtactgcgacaacgccggcagcgtctccttcttcccgcaggccgagacctgcaaggtgcagagcaaccgcgtgttctgcgacaccatgaactccctgacgctgcccagcgagatcaacctctgcaacgtcgacatcttcaaccccaagtacgactgcaagatcatgacctccaagaccgacgtgagctccagcgtgatcacctccctgggggccatcgtcagctgctacggcaagacgaagtgcaccgccagcaacaagaaccgggggatcatcaagaccttctccaacggctgcgactacgtgagcaacaagggcgtggacaccgtgtccgtcgggaacaccctgtactacgtgaacaagcaggagggcaagagcctctacgtgaagggggagcccatcatcaacttctacgacccgctggtcttcccctccgacgagttcgacgcgagcatctcccaggtgaacgagaagatcaaccagagcctggccttcatccgcaagtccgacgagctgctccacaacgtgaacgccggcaagagcacgaccaacatcatgatcaccaccatcatcatcgtcatcatcgtgatcctgctgtccctcatcgccgtggggctgctgctctactgcaaggcccggagcacgcccgtcaccctgtccaaggaccagctgagcggcatcaacaacatcgcgttctccaactga

SEQ ID NO: 18 - RNA, 1698 nt, synthetic construct
  misc_feature 1..1698: note = GC-enriched RNA sequence without UTRs coding for the Hemagglutinin (HA) protein of Influenza A/Puerto Rico/8/1934
  source 1..1698: mol_type = other RNA
atgaaggccaacctgctcgtgctgctgtgcgccctcgcggccgccgacgccgacaccatctgcatcggctaccacgccaacaacagcaccgacacggtcgacaccgtgctggagaagaacgtgaccgtcacccactccgtgaacctgctcgaggacagccacaacgggaagctgtgccggctgaagggcatcgcgcccctccagctggggaagtgcaacatcgccggctggctgctcgggaacccggagtgcgaccccctgctgcccgtgcgctcctggagctacatcgtcgagacgcccaactccgagaacggcatctgctacccgggcgacttcatcgactacgaggagctccgggagcagctgagctccgtgagctccttcgagcgcttcgagatcttccccaaggagagctcctggcccaaccacaacaccaacggggtgaccgccgcctgcagccacgagggcaagtccagcttctaccggaacctgctctggctgaccgagaaggaggggtcctaccccaagctgaagaacagctacgtcaacaagaagggcaaggaggtgctcgtgctgtgggggatccaccacccgcccaactccaaggagcagcagaacctgtaccagaacgagaacgcgtacgtcagcgtggtgacgtccaactacaaccgccggttcacccccgagatcgccgagcgccccaaggtccgggaccaggccggccgcatgaactactactggaccctcctgaagccgggcgacaccatcatcttcgaggccaacgggaacctgatcgccccgatgtacgcgttcgccctcagccggggcttcgggagcggcatcatcacgtccaacgccagcatgcacgagtgcaacaccaagtgccagacccccctgggcgccatcaactccagcctgccctaccagaacatccacccggtgaccatcggggagtgccccaagtacgtgcgctccgccaagctccggatggtcacgggcctgcgcaacaaccccagcatccagtcccgggggctgttcggcgcgatcgccgggttcatcgagggcggctggaccgggatgatcgacggctggtacgggtaccaccaccagaacgagcagggcagcgggtacgccgccgaccagaagtccacccagaacgccatcaacggcatcaccaacaaggtgaacacggtgatcgagaagatgaacatccagttcaccgcggtcggcaaggagttcaacaagctcgagaagcgcatggagaacctgaacaagaaggtggacgacgggttcctggacatctggacctacaacgccgagctcctggtgctgctcgagaacgagcggaccctggacttccacgacagcaacgtcaagaacctgtacgagaaggtgaagtcccagctcaagaacaacgccaaggagatcggcaacgggtgcttcgagttctaccacaagtgcgacaacgagtgcatggagagcgtccgcaacggcacgtacgactaccccaagtactccgaggagagcaagctgaaccgggagaaggtggacggggtgaagctggagtccatgggcatctaccagatcctcgccatctacagcaccgtcgcctccagcctggtgctgctggtgtccctcggcgcgatcagcttctggatgtgcagcaacgggtccctgcagtgccgcatctgcatctga

SEQ ID NO: 19 - RNA, 1942 nt, synthetic construct
  misc_feature 1..1942: note = GC-enriched full mRNA sequence coding for the Fusion (F) protein of RSV Long
  source 1..1942: mol_type = other RNA
gggagaaagcttaccatggagctgcccatcctcaaggccaacgccatcaccaccatcctggcggccgtgacgttctgcttcgccagctcccagaacatcaccgaggagttctaccagagcacctgctccgccgtcagcaagggctacctgtccgccctccggaccgggtggtacacgagcgtgatcaccatcgagctgtccaacatcaaggagaacaagtgcaacggcaccgacgcgaaggtgaagctgatcaaccaggagctcgacaagtacaagaacgccgtcaccgagctgcagctgctcatgcagagcacgaccgccgccaacaaccgcgcgcggcgcgagctgccgcggttcatgaactacaccctgaacaacaccaagaagacgaacgtgaccctctccaagaagcgcaagcggcgcttcctggggttcctgctcggcgtggggagcgccatcgcctccggcatcgccgtcagcaaggtgctgcacctggagggcgaggtgaacaagatcaagtccgccctcctgagcaccaacaaggcggtcgtgtccctgagcaacggggtgtccgtcctcaccagcaaggtgctggacctgaagaactacatcgacaagcagctcctgcccatcgtgaacaagcagtcctgccggatcagcaacatcgagacggtcatcgagttccagcagaagaacaaccgcctgctcgagatcacccgggagttcagcgtgaacgccggcgtgaccacccccgtctccacgtacatgctgaccaacagcgagctgctctccctgatcaacgacatgcccatcaccaacgaccagaagaagctgatgagcaacaacgtgcagatcgtgcgccagcagtcctacagcatcatgtccatcatcaaggaggaggtcctcgcctacgtggtgcagctgccgctgtacggggtcatcgacaccccctgctggaagctccacacgagccccctgtgcaccaccaacaccaaggagggctccaacatctgcctgacgcggaccgaccgcgggtggtactgcgacaacgccggcagcgtgtccttcttcccccaggccgagacctgcaaggtccagagcaaccgggtgttctgcgacaccatgaactccctcacgctgccgagcgaggtgaacctgtgcaacgtcgacatcttcaaccccaagtacgactgcaagatcatgacctccaagaccgacgtgagctccagcgtgatcacctccctcggcgcgatcgtcagctgctacgggaagacgaagtgcaccgccagcaacaagaaccgcggcatcatcaagaccttctccaacgggtgcgactacgtgagcaacaagggcgtggacaccgtctccgtgggcaacaccctgtactacgtgaacaagcaggaggggaagagcctgtacgtcaagggcgagcccatcatcaacttctacgaccccctcgtgttcccgtccgacgagttcgacgccagcatctcccaggtgaacgagaagatcaaccagagcctggccttcatccggaagtccgacgagctgctgcaccacgtcaacgccgggaagagcacgaccaacatcatgatcaccaccatcatcatcgtgatcatcgtgatcctcctgtccctgatcgcggtcggcctcctgctgtactgcaaggcccgcagcacgcccgtgaccctctccaaggaccagctgagcgggatcaacaacatcgccttctccaactgaggactagttataagactgactagcccgatgggcctcccaacgggccctcctcccctccttgcaccgagattaataaaaaaaaaaaaaaaaaaaaaaaaaaaaaaaaaaaaaaaaaaaaaaaaaaaaaaaaaaaaaaaatgcatcccccccccccccccccccccccccccccccaaaggctcttttcagagccaccagaatt

SEQ ID NO: 20 - RNA, 1942 nt, synthetic construct
  misc_feature 1..1942: note = GC-enriched full mRNA sequence coding for the Fusion (F) protein of RSV A2
  source 1..1942: mol_type = other RNA
gggagaaagcttaccatggagctgctcatcctgaaggccaacgccatcaccaccatcctgacggcggtgaccttctgcttcgccagcggccagaacatcaccgaggagttctaccagtccacctgcagcgccgtctccaaggggtacctcagcgccctgcggacgggctggtacacctccgtgatcaccatcgagctgagcaacatcaaggagaacaagtgcaacgggaccgacgccaaggtgaagctcatcaagcaggagctggacaagtacaagaacgcggtcacggagctgcagctcctgatgcagtccaccccgccgaccaacaaccgcgcccggcgcgagctgccccggttcatgaactacaccctcaacaacgccaagaagacgaacgtgaccctgagcaagaagcgcaagcggcgcttcctgggcttcctcctgggggtgggctccgccatcgcgagcggcgtcgccgtgtccaaggtgctgcacctcgagggggaggtcaacaagatcaagagcgccctgctgtccaccaacaaggccgtggtgagcctctccaacggcgtcagcgtgctgacctccaaggtgctggacctcaagaactacatcgacaagcagctgctgcccatcgtcaacaagcagagctgctccatcagcaacatcgagacggtgatcgagttccagcagaagaacaaccggctcctggagatcacccgcgagttcagcgtgaacgccggggtcaccacccccgtgtccacgtacatgctgaccaacagcgagctcctgtccctgatcaacgacatgccgatcaccaacgaccagaagaagctcatgagcaacaacgtgcagatcgtccggcagcagtcctacagcatcatgtccatcatcaaggaggaggtgctggcgtacgtggtccagctgcccctctacggcgtgatcgacaccccctgctggaagctgcacacgagccccctgtgcaccaccaacaccaaggaggggtccaacatctgcctcacgcgcaccgaccggggctggtactgcgacaacgccggcagcgtctccttcttcccgcaggccgagacctgcaaggtgcagagcaaccgcgtgttctgcgacaccatgaactccctgacgctgcccagcgagatcaacctctgcaacgtcgacatcttcaaccccaagtacgactgcaagatcatgacctccaagaccgacgtgagctccagcgtgatcacctccctgggggccatcgtcagctgctacggcaagacgaagtgcaccgccagcaacaagaaccgggggatcatcaagaccttctccaacggctgcgactacgtgagcaacaagggcatggacaccgtgtccgtcgggaacaccctgtactacgtgaacaagcaggagggcaagagcctctacgtgaagggggagcccatcatcaacttctacgacccgctggtcttcccctccgacgagttcgacgcgagcatctcccaggtgaacgagaagatcaaccagagcctggccttcatccgcaagtccgacgagctgctccacaacgtgaacgccggcaagagcacgaccaacatcatgatcaccaccatcatcatcgtcatcatcgtgatcctgctgtccctcatcgccgtggggctgctgctctactgcaaggcccggagcacgcccgtcaccctgtccaaggaccagctgagcggcatcaacaacatcgcgttctccaactgaggactagttataagactgactagcccgatgggcctcccaacgggccctcctcccctccttgcaccgagattaataaaaaaaaaaaaaaaaaaaaaaaaaaaaaaaaaaaaaaaaaaaaaaaaaaaaaaaaaaaaaaaatgcatcccccccccccccccccccccccccccccccaaaggctcttttcagagccaccagaatt

SEQ ID NO: 21 - RNA, 1915 nt, synthetic construct
  misc_feature 1..1915: note = GC-enriched full mRNA sequence coding for the Hemagglutinin (HA) protein of Influenza A/Puerto Rico/8/1934
  source 1..1915: mol_type = other RNA
gggagaaagcttaccatgaaggccaacctgctcgtgctgctgtgcgccctcgcggccgccgacgccgacaccatctgcatcggctaccacgccaacaacagcaccgacacggtcgacaccgtgctggagaagaacgtgaccgtcacccactccgtgaacctgctcgaggacagccacaacgggaagctgtgccggctgaagggcatcgcgcccctccagctggggaagtgcaacatcgccggctggctgctcgggaacccggagtgcgaccccctgctgcccgtgcgctcctggagctacatcgtcgagacgcccaactccgagaacggcatctgctacccgggcgacttcatcgactacgaggagctccgggagcagctgagctccgtgagctccttcgagcgcttcgagatcttccccaaggagagctcctggcccaaccacaacaccaacggggtgaccgccgcctgcagccacgagggcaagtccagcttctaccggaacctgctctggctgaccgagaaggaggggtcctaccccaagctgaagaacagctacgtcaacaagaagggcaaggaggtgctcgtgctgtgggggatccaccacccgcccaactccaaggagcagcagaacctgtaccagaacgagaacgcgtacgtcagcgtggtgacgtccaactacaaccgccggttcacccccgagatcgccgagcgccccaaggtccgggaccaggccggccgcatgaactactactggaccctcctgaagccgggcgacaccatcatcttcgaggccaacgggaacctgatcgccccgatgtacgcgttcgccctcagccggggcttcgggagcggcatcatcacgtccaacgccagcatgcacgagtgcaacaccaagtgccagacccccctgggcgccatcaactccagcctgccctaccagaacatccacccggtgaccatcggggagtgccccaagtacgtgcgctccgccaagctccggatggtcacgggcctgcgcaacaaccccagcatccagtcccgggggctgttcggcgcgatcgccgggttcatcgagggcggctggaccgggatgatcgacggctggtacgggtaccaccaccagaacgagcagggcagcgggtacgccgccgaccagaagtccacccagaacgccatcaacggcatcaccaacaaggtgaacacggtgatcgagaagatgaacatccagttcaccgcggtcggcaaggagttcaacaagctcgagaagcgcatggagaacctgaacaagaaggtggacgacgggttcctggacatctggacctacaacgccgagctcctggtgctgctcgagaacgagcggaccctggacttccacgacagcaacgtcaagaacctgtacgagaaggtgaagtcccagctcaagaacaacgccaaggagatcggcaacgggtgcttcgagttctaccacaagtgcgacaacgagtgcatggagagcgtccgcaacggcacgtacgactaccccaagtactccgaggagagcaagctgaaccgggagaaggtggacggggtgaagctggagtccatgggcatctaccagatcctcgccatctacagcaccgtcgcctccagcctggtgctgctggtgtccctcggcgcgatcagcttctggatgtgcagcaacgggtccctgcagtgccgcatctgcatctgaccactagttataagactgactagcccgatgggcctcccaacgggccctcctcccctccttgcaccgagattaataaaaaaaaaaaaaaaaaaaaaaaaaaaaaaaaaaaaaaaaaaaaaaaaaaaaaaaaaaaaaaaatgcatcccccccccccccccccccccccccccccccaaaggctcttttcagagccaccagaatt

SEQ ID NO: 22 - protein, 9 aa, Influenza A virus
YPYDVPDYA

SEQ ID NO: 23 - RNA, 547 nt, synthetic construct
  misc_feature 1..547: note = Non-coding RNA used as a control
  source 1..547: mol_type = other RNA
gggagaaagctcaagcttggagcaatgcccgcacattgaggaaaccgagttgcatatctcagagtattggcccccgtgtaggttattcttgacagacagtggagcttattcactcccaggatccgagtcgcatactacggtactggtgacagacctaggtcgtcagttgaccagtccgccactagacgtgagtccgtcaaagcagttagatgttacactctattagatctcggattacagctggaaggagcaggagtagtgttcttgctctaagtaccgagtgtgcccaatacccgatcagcttattaacgaacggctcctcctcttagactgcagcgtaagtgcggaatctggggatcaaattactgactgcctggattaccctcggacatataaccttgtagcacgctgttgctgtataggtgaccaacgcccactcgagtagaccagctctcttagtccggacaatgataggaggcgcggtcaatctacttctggctagttaagaataggctgcaccgacctctataagtagcgtgtcctctag

SEQ ID NO: 24 - protein, 9 aa, respiratory syncytial virus
KYKNAVTEL

SEQ ID NO: 25 - protein, 10 aa, respiratory syncytial virus
TYMLTNSELL

SEQ ID NO: 26 - protein, 9 aa, respiratory syncytial virus
FPQAETCKV